European Patent Specification EP 3 708 179 B1, published October 4, 2023. Title: Formulations of Guanylate Cyclase C Agonists and Methods of Use. Applicant: Comiskey, Stephen Feng, Rong Foss, John Shailubhai, Kunwar. The sequence listing filed with the application follows.

SEQUENCE LISTING (261 sequences)

SEQ ID NO: 1 - protein, 16 aa, Artificial Sequence
  Chemically Synthesized
NDECELCVNVACTGCL

SEQ ID NO: 2 - protein, 15 aa, Artificial Sequence
  Chemically Synthesized
DECELCVNVACTGCL

SEQ ID NO: 3 - protein, 14 aa, Artificial Sequence
  Chemically Synthesized
DECELCVNVACTGC

SEQ ID NO: 4 - protein, 14 aa, Artificial Sequence
  Chemically Synthesized
ECELCVNVACTGCL

SEQ ID NO: 5 - protein, 13 aa, Artificial Sequence
  Chemically Synthesized
ECELCVNVACTGC

SEQ ID NO: 6 - protein, 13 aa, Artificial Sequence
  Chemically Synthesized
CELCVNVACTGCL

SEQ ID NO: 7 - protein, 12 aa, Artificial Sequence
  Chemically Synthesized
CELCVNVACTGC

SEQ ID NO: 8 - protein, 16 aa, Artificial Sequence
  Chemically Synthesized
  MISC_FEATURE (16)..(16): wherein LEU is a D-amino acid
NDECELCVNVACTGCL

SEQ ID NO: 9 - protein, 16 aa, Artificial Sequence
  Chemically Synthesized
  MISC_FEATURE (1)..(1): wherein ASN is a D-amino acid
  MISC_FEATURE (16)..(16): wherein LEU is a D-amino acid
NDECELCVNVACTGCL

SEQ ID NO: 10 - protein, 16 aa, Artificial Sequence
  Chemically Synthesized
  MISC_FEATURE (1)..(1): wherein ASN is a D-amino acid
  MISC_FEATURE (2)..(2): wherein ASP is a D-amino acid
  MISC_FEATURE (16)..(16): wherein LEU is a D-amino acid
NDECELCVNVACTGCL

SEQ ID NO: 11 - protein, 16 aa, Artificial Sequence
  Chemically Synthesized
  MISC_FEATURE (1)..(1): wherein ASN is a D-amino acid
  MISC_FEATURE (2)..(2): wherein ASP is a D-amino acid
  MISC_FEATURE (3)..(3): wherein GLU is a D-amino acid
  MISC_FEATURE (16)..(16): wherein LEU is a D-amino acid
NDECELCVNVACTGCL

SEQ ID NO: 12 - protein, 16 aa, Artificial Sequence
  Chemically Synthesized
  MISC_FEATURE (1)..(1): wherein ASN is a D-amino acid
NDECELCVNVACTGCL

SEQ ID NO: 13 - protein, 16 aa, Artificial Sequence
  Chemically Synthesized
  MISC_FEATURE (1)..(1): wherein ASN is a D-amino acid
  MISC_FEATURE (6)..(6): wherein LEU is a D-amino acid
  MISC_FEATURE (16)..(16): wherein LEU is a D-amino acid
NDECELCVNVACTGCL

SEQ ID NO: 14 - protein, 15 aa, Artificial Sequence
  Chemically Synthesized
NDECELCVNVACTGC

SEQ ID NO: 15 - protein, 16 aa, Artificial Sequence
  Chemically Synthesized
  MISC_FEATURE (1)..(1): wherein ASN at position 1 is attached to polyethylene glycol
  MISC_FEATURE (16)..(16): wherein LEU is a D-amino acid
  MISC_FEATURE (16)..(16): wherein LEU at position 16 is attached to polyethylene glycol
NDECELCVNVACTGCL

SEQ ID NO: 16 - protein, 16 aa, Artificial Sequence
  Chemically Synthesized
  MISC_FEATURE (1)..(1): wherein ASN at position 1 is attached to polyethylene glycol
  MISC_FEATURE (1)..(1): wherein ASN is a D-amino acid
  MISC_FEATURE (16)..(16): wherein LEU is a D-amino acid
  MISC_FEATURE (16)..(16): wherein LEU at position 16 is attached to polyethylene glycol
NDECELCVNVACTGCL

SEQ ID NO: 17 - protein, 16 aa, Artificial Sequence
  Chemically Synthesized
  MISC_FEATURE (1)..(1): wherein ASN at position 1 is attached to polyethylene glycol
  MISC_FEATURE (1)..(1): wherein ASN is a D-amino acid
  MISC_FEATURE (2)..(2): wherein ASP is a D-amino acid
  MISC_FEATURE (16)..(16): wherein LEU is a D-amino acid
  MISC_FEATURE (16)..(16): wherein LEU at position 16 is attached to polyethylene glycol
NDECELCVNVACTGCL

SEQ ID NO: 18 - protein, 16 aa, Artificial Sequence
  Chemically Synthesized
  MISC_FEATURE (1)..(1): wherein ASN is a D-amino acid
  MISC_FEATURE (16)..(16): wherein LEU at position 16 is attached to polyethylene glycol
  MISC_FEATURE (16)..(16): wherein LEU is a D-amino acid
NDECELCVNVACTGCL

SEQ ID NO: 19 - protein, 16 aa, Artificial Sequence
  Chemically Synthesized
  MISC_FEATURE (1)..(1): wherein ASN at position 1 is attached to polyethylene glycol
  MISC_FEATURE (16)..(16): wherein LEU is a D-amino acid
NDECELCVNVACTGCL

SEQ ID NO: 20 - protein, 16 aa, Artificial Sequence
  Chemically Synthesized
  MISC_FEATURE (1)..(1): wherein ASN at position 1 is attached to polyethylene glycol
  MISC_FEATURE (1)..(1): wherein ASN is a D-amino acid
  MISC_FEATURE (16)..(16): wherein LEU is a D-amino acid
NDECELCVNVACTGCL

SEQ ID NO: 21 - protein, 16 aa, Artificial Sequence
  Chemically Synthesized
  MISC_FEATURE (16)..(16): wherein LEU at position 16 is attached to polyethylene glycol
  MISC_FEATURE (16)..(16): wherein LEU is a D-amino acid
NDECELCVNVACTGCL

SEQ ID NO: 22 - protein, 16 aa, Artificial Sequence
  Chemically Synthesized
  MISC_FEATURE (1)..(1): wherein ASN at position 1 is attached to polyethylene glycol
  MISC_FEATURE (1)..(1): wherein ASN is a D-amino acid
  MISC_FEATURE (2)..(2): wherein ASP is a D-amino acid
  MISC_FEATURE (3)..(3): wherein GLU is a D-amino acid
  MISC_FEATURE (16)..(16): wherein LEU is a D-amino acid
  MISC_FEATURE (16)..(16): wherein LEU at position 16 is attached to polyethylene glycol
NDECELCVNVACTGCL

SEQ ID NO: 23 - protein, 16 aa, Artificial Sequence
  Chemically Synthesized
  MISC_FEATURE (1)..(1): wherein ASN at position 1 is attached to polyethylene glycol
  MISC_FEATURE (1)..(1): wherein ASN is a D-amino acid
  MISC_FEATURE (2)..(2): wherein ASP is a D-amino acid
  MISC_FEATURE (3)..(3): wherein GLU is a D-amino acid
  MISC_FEATURE (16)..(16): wherein LEU is a D-amino acid
NDECELCVNVACTGCL

SEQ ID NO: 24 - protein, 16 aa, Artificial Sequence
  Chemically Synthesized
  MISC_FEATURE (1)..(1): wherein ASN is a D-amino acid
  MISC_FEATURE (2)..(2): wherein ASP is a D-amino acid
  MISC_FEATURE (3)..(3): wherein GLU is a D-amino acid
  MISC_FEATURE (16)..(16): wherein LEU at position 16 is attached to polyethylene glycol
  MISC_FEATURE (16)..(16): wherein LEU is a D-amino acid
NDECELCVNVACTGCL

SEQ ID NO: 25 - protein, 16 aa, Artificial Sequence
  Chemically Synthesized
  MISC_FEATURE (1)..(1): wherein ASN is a D-amino acid
  MISC_FEATURE (2)..(2): wherein ASP is a D-amino acid
  MISC_FEATURE (16)..(16): wherein LEU at position 16 is attached to polyethylene glycol
  MISC_FEATURE (16)..(16): wherein LEU is a D-amino acid
NDECELCVNVACTGCL

SEQ ID NO: 26 - protein, 16 aa, Artificial Sequence
  Chemically Synthesized
  MISC_FEATURE (1)..(1): wherein ASN at position 1 is attached to polyethylene glycol
  MISC_FEATURE (1)..(1): wherein ASN is a D-amino acid
  MISC_FEATURE (2)..(2): wherein ASP is a D-amino acid
  MISC_FEATURE (16)..(16): wherein LEU is a D-amino acid
NDECELCVNVACTGCL

SEQ ID NO: 27 - protein, 16 aa, Artificial Sequence
  Chemically Synthesized
  MISC_FEATURE (1)..(1): wherein ASN is a D-amino acid
  MISC_FEATURE (16)..(16): wherein x is 3-(2-naphthyl)alanine
  MISC_FEATURE (16)..(16): wherein x is a D-amino acid
NDECELCVNVACTGCX

SEQ ID NO: 28 - protein, 16 aa, Artificial Sequence
  Chemically Synthesized
  MISC_FEATURE (1)..(1): wherein ASN is a D-amino acid
  MOD_RES (8)..(8): wherein the x is a 2-aminoisobutyric acid, Aib
  MOD_RES (10)..(10): wherein the x is a 2-aminoisobutyric acid, Aib
  MISC_FEATURE (16)..(16): wherein LEU is a D-amino acid
NDECELCXNXACTGCL

SEQ ID NO: 29 - protein, 16 aa, Artificial Sequence
  Chemically Synthesized
  MISC_FEATURE (1)..(1): wherein ASN is a D-amino acid
  MISC_FEATURE (7)..(7): wherein ASP at position 7 is attached to a Lactam bridge
  MISC_FEATURE (15)..(15): wherein x at position 15 is ornithine
  MOD_RES (15)..(15): wherein x is an ornithine, Orn
  MISC_FEATURE (16)..(16): wherein LEU is a D-amino acid
NDECELDVNVACTGXL

SEQ ID NO: 30 - protein, 16 aa, Artificial Sequence
  Chemically Synthesized
  MISC_FEATURE (1)..(1): wherein ASN is a D-amino acid
  MISC_FEATURE (16)..(16): wherein LEU is a D-amino acid
NDECEYCVNVACTGCL

SEQ ID NO: 31 - protein, 16 aa, Artificial Sequence
  Chemically Synthesized
  MISC_FEATURE (1)..(1): wherein ASN is a D-amino acid
  MISC_FEATURE (16)..(16): wherein LEU is a D-amino acid
NDECESCVNVACTGCL

SEQ ID NO: 32 - protein, 16 aa, Artificial Sequence
  Chemically Synthesized
  MISC_FEATURE (1)..(1): wherein ASN at position 1 is attached to polyethylene glycol
  MISC_FEATURE (1)..(1): wherein ASN is a D-amino acid
  MISC_FEATURE (16)..(16): wherein LEU is a D-amino acid
  MISC_FEATURE (16)..(16): wherein LEU at position 16 is attached to polyethylene glycol
NDECEYCVNVACTGCL

SEQ ID NO: 33 - protein, 16 aa, Artificial Sequence
  Chemically Synthesized
  MISC_FEATURE (1)..(1): wherein ASN at position 1 is attached to polyethylene glycol
  MISC_FEATURE (1)..(1): wherein ASN is a D-amino acid
  MISC_FEATURE (16)..(16): wherein LEU is a D-amino acid
NDECEYCVNVACTGCL

SEQ ID NO: 34 - protein, 16 aa, Artificial Sequence
  Chemically Synthesized
  MISC_FEATURE (1)..(1): wherein ASN is a D-amino acid
  MISC_FEATURE (16)..(16): wherein LEU at position 16 is attached to polyethylene glycol
  MISC_FEATURE (16)..(16): wherein LEU is a D-amino acid
NDECEYCVNVACTGCL

SEQ ID NO: 35 - protein, 16 aa, Artificial Sequence
  Chemically Synthesized
  MISC_FEATURE (1)..(1): wherein ASN at position 1 is attached to polyethylene glycol
  MISC_FEATURE (1)..(1): wherein ASN is a D-amino acid
  MISC_FEATURE (16)..(16): wherein LEU is a D-amino acid
  MISC_FEATURE (16)..(16): wherein LEU at position 16 is attached to polyethylene glycol
NDECESCVNVACTGCL

SEQ ID NO: 36 - protein, 16 aa, Artificial Sequence
  Chemically Synthesized
  MISC_FEATURE (1)..(1): wherein ASN at position 1 is attached to polyethylene glycol
  MISC_FEATURE (1)..(1): wherein ASN is a D-amino acid
  MISC_FEATURE (16)..(16): wherein LEU is a D-amino acid
NDECESCVNVACTGCL

SEQ ID NO: 37 - protein, 16 aa, Artificial Sequence
  Chemically Synthesized
  MISC_FEATURE (1)..(1): wherein ASN is a D-amino acid
  MISC_FEATURE (16)..(16): wherein LEU at position 16 is attached to polyethylene glycol
  MISC_FEATURE (16)..(16): wherein LEU is a D-amino acid
NDECESCVNVACTGCL

SEQ ID NO: 38 - protein, 16 aa, Artificial Sequence
  Chemically Synthesized
NDECELCVNVACTGCS

SEQ ID NO: 39 - protein, 16 aa, Artificial Sequence
  Chemically Synthesized
  MISC_FEATURE (1)..(1): wherein ASN at position 1 is attached to polyethylene glycol
  MISC_FEATURE (16)..(16): wherein SER at position 16 is attached to polyethylene glycol
NDECELCVNVACTGCS

SEQ ID NO: 40 - protein, 16 aa, Artificial Sequence
  Chemically Synthesized
  MISC_FEATURE (1)..(1): wherein ASN at position 1 is attached to polyethylene glycol
NDECELCVNVACTGCS

SEQ ID NO: 41 - protein, 16 aa, Artificial Sequence
  Chemically Synthesized
  MISC_FEATURE (16)..(16): wherein SER at position 16 is attached to polyethylene glycol
NDECELCVNVACTGCS

SEQ ID NO: 42 - protein, 16 aa, Artificial Sequence
  Chemically Synthesized
  MISC_FEATURE (1)..(1): wherein ASN at position 1 is attached to polyethylene glycol
  MISC_FEATURE (16)..(16): wherein SER is a D-amino acid
  MISC_FEATURE (16)..(16): wherein SER at position 16 is attached to polyethylene glycol
NDECELCVNVACTGCS

SEQ ID NO: 43 - protein, 16 aa, Artificial Sequence
  Chemically Synthesized
  MISC_FEATURE (1)..(1): wherein ASN at position 1 is attached to polyethylene glycol
  MISC_FEATURE (16)..(16): wherein SER is a D-amino acid
NDECELCVNVACTGCS

SEQ ID NO: 44 - protein, 16 aa, Artificial Sequence
  Chemically Synthesized
  MISC_FEATURE (16)..(16): wherein SER at position 16 is attached to polyethylene glycol
  MISC_FEATURE (16)..(16): wherein SER is a D-amino acid
NDECELCVNVACTGCS

SEQ ID NO: 45 - protein, 16 aa, Artificial Sequence
  Chemically Synthesized
  MISC_FEATURE (5)..(6): wherein x is any natural, or unnatural amino acid or amino acid analogue, and may be an L-amino acid, or a D-amino acid, or a methylated or an unmethylated amino acid
  MISC_FEATURE (8)..(11): wherein x is any natural, or unnatural amino acid or amino acid analogue, and may be an L-amino acid, or a D-amino acid, or a methylated or an unmethylated amino acid
  MISC_FEATURE (13)..(14): wherein x is any natural, or unnatural amino acid or amino acid analogue, and may be an L-amino acid, or a D-amino acid, or a methylated or an unmethylated amino acid
  MISC_FEATURE (16)..(16): wherein x is any natural, or unnatural amino acid or amino acid analogue, and may be an L-amino acid, or a D-amino acid, or a methylated or an unmethylated amino acid
NDECXXCXXXXCXXCX

SEQ ID NO: 46 - protein, 16 aa, Artificial Sequence
  Chemically Synthesized
  MISC_FEATURE (1)..(1): wherein x is any natural, or unnatural amino acid or amino acid analogue and may be an L-amino acid, or a D-amino acid, or a methylated or an unmethylated amino acid
  MISC_FEATURE (2)..(2): wherein x is any natural, or unnatural amino acid or amino acid analogue that is zero or one residue in length and may be an L-amino acid, or a D-amino acid, or a methylated or an unmethylated amino acid
  MISC_FEATURE (3)..(3): wherein x is any natural, or unnatural amino acid or amino acid analogue that is zero or one residue in length and may be an L-amino acid, or a D-amino acid, or a methylated or an unmethylated amino acid
  MISC_FEATURE (5)..(6): wherein x is any natural, or unnatural amino acid, or amino acid analogue and may be an L-amino acid, or a D-amino acid, or a methylated or an unmethylated amino acid
  MISC_FEATURE (8)..(11): wherein x is any natural, or unnatural amino acid, or amino acid analogue and may be an L-amino acid, or a D-amino acid, or a methylated or an unmethylated amino acid
  MISC_FEATURE (13)..(14): wherein x is any natural, or unnatural amino acid, or amino acid analogue and may be an L-amino acid, or a D-amino acid, or a methylated or an unmethylated amino acid
  MISC_FEATURE (16)..(16): wherein x is any natural, or unnatural amino acid, or amino acid analogue that is zero or one residue in length and may be an L-amino acid, or a D-amino acid, or a methylated or an unmethylated amino acid
XXXCXXCXXXXCXXCX

SEQ ID NO: 47 - protein, 16 aa, Artificial Sequence
  Chemically Synthesized
  MISC_FEATURE (1)..(1): wherein x is any natural, or unnatural amino acid or amino acid analogue and may be an L-amino acid, or a D-amino acid, or a methylated or an unmethylated amino acid
  MISC_FEATURE (2)..(2): wherein x is any natural, or unnatural amino acid or amino acid analogue that is zero or one residue in length and may be an L-amino acid, or a D-amino acid, or a methylated or an unmethylated amino acid
  MISC_FEATURE (3)..(3): wherein x is any natural, or unnatural amino acid or amino acid analogue that is zero or one residue in length and may be an L-amino acid, or a D-amino acid, or a methylated or an unmethylated amino acid
  MISC_FEATURE (4)..(4): wherein x is a cysteine, penicillamine homocysteine, or 3-mercaptoproline
  MISC_FEATURE (6)..(6): wherein x is any natural, or unnatural amino acid, or amino acid analogue and may be an L-amino acid, or a D-amino acid, or a methylated or an unmethylated amino acid
  MISC_FEATURE (7)..(7): wherein x is a cysteine, penicillamine homocysteine, or 3-mercaptoproline
  MISC_FEATURE (12)..(12): wherein x is a cysteine, penicillamine homocysteine, or 3-mercaptoproline
  MISC_FEATURE (15)..(15): wherein x is a cysteine, penicillamine homocysteine, or 3-mercaptoproline
  MISC_FEATURE (16)..(16): wherein x is any natural, or unnatural amino acid or amino acid analogue that is zero or one residue in length and may be an L-amino acid, or a D-amino acid, or a methylated or an unmethylated amino acid
XXXXEXXVNVAXTGXX

SEQ ID NO: 48 - protein, 16 aa, Artificial Sequence
  Chemically Synthesized
  MISC_FEATURE (1)..(1): wherein x is any natural, or unnatural amino acid or amino acid analogue and may be an L-amino acid, or a D-amino acid, or a methylated or an unmethylated amino acid
  MISC_FEATURE (2)..(2): wherein x is any natural, or unnatural amino acid or amino acid analogue that is zero or one residue in length and may be an L-amino acid, or a D-amino acid, or a methylated or an unmethylated amino acid
  MISC_FEATURE (3)..(3): wherein x is any natural, or unnatural amino acid or amino acid analogue that is zero or one residue in length and may be an L-amino acid, or a D-amino acid, or a methylated or an unmethylated amino acid
  MISC_FEATURE (4)..(4): wherein x is a cysteine, penicillamine homocysteine, or 3-mercaptoproline
  MISC_FEATURE (5)..(6): wherein x is any natural, or unnatural amino acid or amino acid analogue and may be an L-amino acid, or a D-amino acid, or a methylated or an unmethylated amino acid
  MISC_FEATURE (7)..(7): wherein x is a cysteine, penicillamine homocysteine, or 3-mercaptoproline
  MISC_FEATURE (8)..(11): wherein x is any natural, or unnatural amino acid or amino acid analogue and may be an L-amino acid, or a D-amino acid, or a methylated or an unmethylated amino acid
  MISC_FEATURE (12)..(12): wherein x is a cysteine, penicillamine homocysteine, or 3-mercaptoproline
  MISC_FEATURE (13)..(14): wherein x is any natural, or unnatural amino acid or amino acid analogue and may be an L-amino acid, or a D-amino acid, or a methylated or an unmethylated amino acid
  MISC_FEATURE (15)..(15): wherein x is a cysteine, penicillamine homocysteine, or 3-mercaptoproline
  MISC_FEATURE (16)..(16): wherein x is any natural, or unnatural amino acid, or amino acid analogue that is zero or one residue in length and may be an L-amino acid, or a D-amino acid, or a methylated or an unmethylated amino acid
XXXXXXXXXXXXXXXX

SEQ ID NO: 49 - protein, 16 aa, Artificial Sequence
  Chemically Synthesized
  MISC_FEATURE (5)..(6): wherein x is any natural, or unnatural amino acid or amino acid analogue and may be an L-amino acid, or a D-amino acid, or a methylated or an unmethylated amino acid
  MISC_FEATURE (8)..(8): wherein x is any natural, or unnatural amino acid or amino acid analogue and may be an L-amino acid, or a D-amino acid, or a methylated or an unmethylated amino acid
  MISC_FEATURE (10)..(11): wherein x is any natural, or unnatural amino acid or amino acid analogue and may be an L-amino acid, or a D-amino acid, or a methylated or an unmethylated amino acid
  MISC_FEATURE (13)..(14): wherein x is any natural, or unnatural amino acid or amino acid analogue and may be an L-amino acid, or a D-amino acid, or a methylated or an unmethylated amino acid
  MISC_FEATURE (16)..(16): wherein x is any natural, or unnatural amino acid or amino acid analogue and may be an L-amino acid, or a D-amino acid, or a methylated or an unmethylated amino acid
NDDCXXCXNXXCXXCX

SEQ ID NO: 50 - protein, 16 aa, Artificial Sequence
  Chemically Synthesized
  MISC_FEATURE (1)..(1): wherein ASN is a D-amino acid
  MISC_FEATURE (5)..(6): wherein x is any natural, or unnatural amino acid, or amino acid analogue and may be an L-amino acid, or a D-amino acid, or a methylated or an unmethylated amino acid
  MISC_FEATURE (8)..(8): wherein x is any natural, or unnatural amino acid or amino acid analogue and may be an L-amino acid, or a D-amino acid, or a methylated or an unmethylated amino acid
  MISC_FEATURE (10)..(11): wherein x is any natural, or unnatural amino acid or amino acid analogue and may be an L-amino acid, or a D-amino acid, or a methylated or an unmethylated amino acid
  MISC_FEATURE (13)..(14): wherein x is any natural, or unnatural amino acid or amino acid analogue and may be an L-amino acid, or a D-amino acid, or a methylated or an unmethylated amino acid
  MISC_FEATURE (16)..(16): wherein x is any natural, or unnatural amino acid, or amino acid analogue and may be an L-amino acid, or a D-amino acid, or a methylated or an unmethylated amino acid
NEECXXCXNXXCXXCX

SEQ ID NO: 51 - protein, 16 aa, Artificial Sequence
  Chemically Synthesized
  MISC_FEATURE (1)..(1): wherein ASN is a D-amino acid
  MISC_FEATURE (2)..(2): wherein GLU is a D-amino acid
  MISC_FEATURE (5)..(6): wherein x is any natural, or unnatural amino acid, or amino acid analogue and may be an L-amino acid, or a D-amino acid, or a methylated or an unmethylated amino acid
  MISC_FEATURE (8)..(8): wherein x is any natural, or unnatural amino acid, or amino acid analogue and may be an L-amino acid, or a D-amino acid, or a methylated or an unmethylated amino acid
  MISC_FEATURE (10)..(11): wherein x is any natural, or unnatural amino acid, or amino acid analogue and may be an L-amino acid, or a D-amino acid, or a methylated or an unmethylated amino acid
  MISC_FEATURE (13)..(14): wherein x is any natural, or unnatural amino acid, or amino acid analogue and may be an L-amino acid, or a D-amino acid, or a methylated or an unmethylated amino acid
  MISC_FEATURE (16)..(16): wherein x is any natural, or unnatural amino acid, or amino acid analogue and may be an L-amino acid, or a D-amino acid, or a methylated or an unmethylated amino acid
NEDCXXCXNXXCXXCX

SEQ ID NO: 52 - protein, 16 aa, Artificial Sequence
  Chemically Synthesized
  MISC_FEATURE (1)..(1): wherein ASN is a D-amino acid
  MISC_FEATURE (2)..(2): wherein ASP is a D-amino acid
  MISC_FEATURE (5)..(6): wherein x is any natural, or unnatural amino acid, or amino acid analogue and may be an L-amino acid, or a D-amino acid, or a methylated or an unmethylated amino acid
  MISC_FEATURE (8)..(8): wherein x is any natural, or unnatural amino acid, or amino acid analogue and may be an L-amino acid, or a D-amino acid, or a methylated or an unmethylated amino acid
  MISC_FEATURE (10)..(11): wherein x is any natural, or unnatural amino acid, or amino acid analogue and may be an L-amino acid, or a D-amino acid, or a methylated or an unmethylated amino acid
  MISC_FEATURE (13)..(14): wherein x is any natural, or unnatural amino acid, or amino acid analogue and may be an L-amino acid, or a D-amino acid, or a methylated or an unmethylated amino acid
  MISC_FEATURE (16)..(16): wherein x is any natural, or unnatural amino acid, or amino acid analogue and may be an L-amino acid, or a D-amino acid, or a methylated or an unmethylated amino acid
NDECXXCXNXXCXXCX

SEQ ID NO: 53 - protein, 16 aa, Artificial Sequence
  Chemically Synthesized
  MISC_FEATURE (1)..(1): wherein ASN is a D-amino acid
  MISC_FEATURE (2)..(2): wherein ASP is a D-amino acid
  MISC_FEATURE (3)..(3): wherein GLU is a D-amino acid
  MISC_FEATURE (5)..(6): wherein x is any natural, or unnatural amino acid, or amino acid analogue and may be an L-amino acid, or a D-amino acid, or a methylated or an unmethylated amino acid
  MISC_FEATURE (8)..(8): wherein x is any natural, or unnatural amino acid, or amino acid analogue and may be an L-amino acid, or a D-amino acid, or a methylated or an unmethylated amino acid
  MISC_FEATURE (10)..(11): wherein x is any natural, or unnatural amino acid, or amino acid analogue and may be an L-amino acid, or a D-amino acid, or a methylated or an unmethylated amino acid
  MISC_FEATURE (13)..(14): wherein x is any natural, or unnatural amino acid, or amino acid analogue and may be an L-amino acid, or a D-amino acid, or a methylated or an unmethylated amino acid
  MISC_FEATURE (16)..(16): wherein x is any natural, or unnatural amino acid, or amino acid analogue and may be an L-amino acid, or a D-amino acid, or a methylated or an unmethylated amino acid
NDECXXCXYXXCXXCX

SEQ ID NO: 54 - protein, 16 aa, Artificial Sequence
  Chemically Synthesized
  MISC_FEATURE (1)..(1): wherein ASN is a D-amino acid
  MISC_FEATURE (2)..(2): wherein GLU is a D-amino acid
  MISC_FEATURE (3)..(3): wherein GLU is a D-amino acid
  MISC_FEATURE (5)..(6): wherein x is any natural, or unnatural amino acid, or amino acid analogue and may be an L-amino acid, or a D-amino acid, a methylated or an unmethylated amino acid
  MISC_FEATURE (8)..(8): wherein x is any natural, or unnatural amino acid, or amino acid analogue and may be an L-amino acid, or a D-amino acid, a methylated or an unmethylated amino acid
  MISC_FEATURE (10)..(11): wherein x is any natural, or unnatural amino acid, or amino acid analogue and may be an L-amino acid, or a D-amino acid, a methylated or an unmethylated amino acid
  MISC_FEATURE (13)..(14): wherein x is any natural, or unnatural amino acid, or amino acid analogue and may be an L-amino acid, or a D-amino acid, a methylated or an unmethylated amino acid
  MISC_FEATURE (16)..(16): wherein x is any natural, or unnatural amino acid, or amino acid analogue and may be an L-amino acid, or a D-amino acid, a methylated or an unmethylated amino acid
NEECXXCXYXXCXXCX

SEQ ID NO: 55 - protein, 14 aa, Artificial Sequence
  Chemically Synthesized
CCEYCCNPACTGCY

SEQ ID NO: 56 - protein, 13 aa, Artificial Sequence
  Chemically Synthesized
CCEYCCNPACTGC

SEQ ID NO: 57 - protein, 14 aa, Artificial Sequence
  Chemically Synthesized
  MISC_FEATURE (1)..(1): wherein CYS at position 1 is attached to polyethylene glycol
  MISC_FEATURE (14)..(14): wherein TYR at position 14 is attached to polyethylene glycol
CCEYCCNPACTGCY

SEQ ID NO: 58 - protein, 16 aa, Artificial Sequence
  Chemically Synthesized
NFCCESCCNPACTGCY

SEQ ID NO: 59 - protein, 16 aa, Artificial Sequence
  Chemically Synthesized
NFCCEFCCNPACTGCY

SEQ ID NO: 60 - protein, 14 aa, Artificial Sequence
  Chemically Synthesized
  MISC_FEATURE (14)..(14): wherein TYR is a D-amino acid
CCEYCCNPACTGCY

SEQ ID NO: 61 - protein, 14 aa, Artificial Sequence
  Chemically Synthesized
  MISC_FEATURE (1)..(1): wherein CYS at position 1 is attached to polyethylene glycol
CCEYCCNPACTGCY

SEQ ID NO: 62 - protein, 16 aa, Artificial Sequence
  Chemically Synthesized
NFCCETCCNPACTGCY

SEQ ID NO: 63 - protein, 16 aa, Artificial Sequence
  Chemically Synthesized
  MISC_FEATURE (16)..(16): wherein TYR is a D-amino acid
NFCCESCCNPACTGCY

SEQ ID NO: 64 - protein, 16 aa, Artificial Sequence
  Chemically Synthesized
  MISC_FEATURE (1)..(1): wherein ASN is a D-amino acid
NFCCESCCNPACTGCY

SEQ ID NO: 65 - protein, 16 aa, Artificial Sequence
  Chemically Synthesized
  MISC_FEATURE (1)..(1): wherein ASN is a D-amino acid
  MISC_FEATURE (16)..(16): wherein TYR is a D-amino acid
NFCCESCCNPACTGCY

SEQ ID NO: 66 - protein, 16 aa, Artificial Sequence
  Chemically Synthesized
  MISC_FEATURE (16)..(16): wherein TYR is a D-amino acid
NFCCETCCNPACTGCY

SEQ ID NO: 67 - protein, 16 aa, Artificial Sequence
  Chemically Synthesized
  MISC_FEATURE (1)..(1): wherein ASN is a D-amino acid
NFCCETCCNPACTGCY

SEQ ID NO: 68 - protein, 16 aa, Artificial Sequence
  Chemically Synthesized
  MISC_FEATURE (1)..(1): wherein ASN is a D-amino acid
  MISC_FEATURE (16)..(16): wherein TYR is a D-amino acid
NFCCETCCNPACTGCY

SEQ ID NO: 69 - protein, 16 aa, Artificial Sequence
  Chemically Synthesized
  MISC_FEATURE (16)..(16): wherein TYR is a D-amino acid
NFCCEFCCNPACTGCY

SEQ ID NO: 70 - protein, 16 aa, Artificial Sequence
  Chemically Synthesized
  MISC_FEATURE (1)..(1): wherein ASN is a D-amino acid
NFCCEFCCNPACTGCY

SEQ ID NO: 71 - protein, 16 aa, Artificial Sequence
  Chemically Synthesized
  MISC_FEATURE (1)..(1): wherein ASN is a D-amino acid
  MISC_FEATURE (16)..(16): wherein TYR is a D-amino acid
NFCCEFCCNPACTGCY

SEQ ID NO: 72 - protein, 14 aa, Artificial Sequence
  Chemically Synthesized
  MISC_FEATURE (14)..(14): wherein TYR at position 14 is attached to polyethylene glycol
CCEYCCNPACTGCY

SEQ ID NO: 73 - protein, 13 aa, Artificial Sequence
  Chemically Synthesized
  MISC_FEATURE (1)..(1): wherein CYS at position 1 is attached to polyethylene glycol
  MISC_FEATURE (13)..(13): wherein CYS at position 13 is attached to polyethylene glycol
CCEYCCNPACTGC

SEQ ID NO: 74 - protein, 13 aa, Artificial Sequence
  Chemically Synthesized
  MISC_FEATURE (1)..(1): wherein CYS at position 1 is attached to polyethylene glycol
CCEYCCNPACTGC

SEQ ID NO: 75 - protein, 13 aa, Artificial Sequence
  Chemically Synthesized
  MISC_FEATURE (13)..(13): wherein CYS at position 13 is attached to polyethylene glycol
CCEYCCNPACTGC

SEQ ID NO: 76 - protein, 16 aa, Artificial Sequence
  Chemically Synthesized
  MISC_FEATURE (1)..(1): wherein ASN at position 1 is attached to polyethylene glycol
  MISC_FEATURE (16)..(16): wherein TYR at position 16 is attached to polyethylene glycol
NFCCESCCNPACTGCY

SEQ ID NO: 77 - protein, 16 aa, Artificial Sequence
  Chemically Synthesized
  MISC_FEATURE (1)..(1): wherein ASN at position 1 is attached to polyethylene glycol
NFCCESCCNPACTGCY

SEQ ID NO: 78 - protein, 16 aa, Artificial Sequence
  Chemically Synthesized
  MISC_FEATURE (16)..(16): wherein TYR at position 16 is attached to polyethylene glycol
NFCCESCCNPACTGCY

SEQ ID NO: 79 - protein, 16 aa, Artificial Sequence
  Chemically Synthesized
  MISC_FEATURE (1)..(1): wherein ASN at position 1 is attached to polyethylene glycol
  MISC_FEATURE (16)..(16): wherein TYR at position 16 is attached to polyethylene glycol
NFCCEFCCNPACTGCY

SEQ ID NO: 80 - protein, 16 aa, Artificial Sequence
  Chemically Synthesized
  MISC_FEATURE (1)..(1): wherein ASN at position 1 is attached to polyethylene glycol
NFCCEFCCNPACTGCY

SEQ ID NO: 81 - protein, 16 aa, Artificial Sequence
  Chemically Synthesized
  MISC_FEATURE (16)..(16): wherein TYR at position 16 is attached to polyethylene glycol
NFCCEFCCNPACTGCY

SEQ ID NO: 82 - protein, 16 aa, Artificial Sequence
  Chemically Synthesized
  MISC_FEATURE (1)..(1): wherein ASN at position 1 is attached to polyethylene glycol
  MISC_FEATURE (16)..(16): wherein TYR at position 16 is attached to polyethylene glycol
NFCCEYCCNPACTGCY

SEQ ID NO: 83 - protein, 16 aa, Artificial Sequence
  Chemically Synthesized
  MISC_FEATURE (1)..(1): wherein ASN at position 1 is attached to polyethylene glycol
NFCCEYCCNPACTGCY

SEQ ID NO: 84 - protein, 16 aa, Artificial Sequence
  Chemically Synthesized
  MISC_FEATURE (16)..(16): wherein TYR at position 16 is attached to polyethylene glycol
NFCCEYCCNPACTGCY

SEQ ID NO: 85 - protein, 14 aa, Artificial Sequence
  Chemically Synthesized
CCESCCNPACTGCY

SEQ ID NO: 86 - protein, 14 aa, Artificial Sequence
  Chemically Synthesized
CCEFCCNPACTGCY

SEQ ID NO: 87 - protein, 13 aa, Artificial Sequence
  Chemically Synthesized
CCESCCNPACTGC

SEQ ID NO: 88 - protein, 13 aa, Artificial Sequence
  Chemically Synthesized
CCEFCCNPACTGC

SEQ ID NO: 89 - protein, 14 aa, Artificial Sequence
  Chemically Synthesized
  MISC_FEATURE (1)..(2): wherein x is penicillamine
  MISC_FEATURE (5)..(6): wherein x is penicillamine
  MISC_FEATURE (10)..(10): wherein x is penicillamine
  MISC_FEATURE (13)..(13): wherein x is penicillamine
XXEYXXNPAXTGXY

SEQ ID NO: 90 - protein, 13 aa, Artificial Sequence
  Chemically Synthesized
  MISC_FEATURE (1)..(2): wherein x is penicillamine
  MISC_FEATURE (5)..(6): wherein x is penicillamine
  MISC_FEATURE (10)..(10): wherein x is penicillamine
  MISC_FEATURE (13)..(13): wherein x is penicillamine
XXEYXXNPAXTGX

SEQ ID NO: 91 - protein, 22 aa, Artificial Sequence
  Chemically Synthesized
  MISC_FEATURE (1)..(6): wherein x is any natural, or unnatural amino acid or amino acid analogue and may be an L-amino acid, or a D-amino acid, or a methylated or an unmethylated amino acid
  MISC_FEATURE (11)..(11): wherein x is any natural, or unnatural amino acid or amino acid analogue and may be an L-amino acid, or a D-amino acid, or a methylated or an unmethylated amino acid
  MISC_FEATURE (15)..(17): wherein x is any natural, or unnatural amino acid or amino acid analogue and may be an L-amino acid, or a D-amino acid, or a methylated or an unmethylated amino acid
  MISC_FEATURE (19)..(20): wherein x is any natural, or unnatural amino acid or amino acid analogue and may be an L-amino acid, or a D-amino acid, or a methylated or an unmethylated amino acid
  MISC_FEATURE (22)..(22): wherein x is any natural, or unnatural amino acid or amino acid analogue and may be an L-amino acid, or a D-amino acid, or a methylated or an unmethylated amino acid
XXXXXXNYCCXYCCXXXCXXCX

SEQ ID NO: 92 - protein, 22 aa, Artificial Sequence
  Chemically Synthesized
  MISC_FEATURE (1)..(6): wherein x is any natural, or unnatural amino acid or amino acid analogue and may be an L-amino acid, or a D-amino acid, or a methylated or an unmethylated amino acid
  MISC_FEATURE (11)..(11): wherein x is any natural, or unnatural amino acid or amino acid analogue and may be an L-amino acid, or a D-amino acid, or a methylated or an unmethylated amino acid
  MISC_FEATURE (15)..(17): wherein x is any natural, or unnatural amino acid or amino acid analogue and may be an L-amino acid, or a D-amino acid, or a methylated or an unmethylated amino acid
  MISC_FEATURE (19)..(20): wherein x is any natural, or unnatural amino acid or amino acid analogue and may be an L-amino acid, or a D-amino acid, or a methylated or an unmethylated amino acid
  MISC_FEATURE (22)..(22): wherein x is any natural, or unnatural amino acid or amino acid analogue and may be an L-amino acid, or a D-amino acid, or a methylated or an unmethylated amino acid
XXXXXXNFCCXFCCXXXCXXCX

SEQ ID NO: 93 - protein, 16 aa, Artificial Sequence
  Chemically Synthesized
  MISC_FEATURE (5)..(5): wherein x is any natural, or unnatural amino acid or amino acid analogue and may be an L-amino acid, or a D-amino acid, or a methylated or an unmethylated amino acid
  MISC_FEATURE (9)..(11): wherein x is any natural, or unnatural amino acid or amino acid analogue and may be an L-amino acid, or a D-amino acid, or a methylated or an unmethylated amino acid
  MISC_FEATURE (13)..(14): wherein x is any natural, or unnatural amino acid or amino acid analogue and may be an L-amino acid, or a D-amino acid, or a methylated or an unmethylated amino acid
  MISC_FEATURE (16)..(16): wherein x is any natural, or unnatural amino acid or amino acid analogue and may be an L-amino acid, or a D-amino acid, or a methylated or an unmethylated amino acid
NFCCXFCCXXXCXXCX

SEQ ID NO: 94 - protein, 16 aa, Artificial Sequence
  Chemically Synthesized
  MISC_FEATURE (3)..(3): wherein x is penicillamine
  MISC_FEATURE (5)..(5): wherein x is any natural, or unnatural amino acid or amino acid analogue and may be an L-amino acid, or a D-amino acid, or a methylated or an unmethylated amino acid
  MISC_FEATURE (8)..(8): wherein x is penicillamine
  MISC_FEATURE (9)..(11): wherein x is any natural, or unnatural amino acid or amino acid analogue and may be an L-amino acid, or a D-amino acid, or a methylated or an unmethylated amino acid
  MISC_FEATURE (13)..(14): wherein x is any natural, or unnatural amino acid or amino acid analogue and may be an L-amino acid, or a D-amino acid, or a methylated or an unmethylated amino acid
  MISC_FEATURE (16)..(16): wherein x is any natural, or unnatural amino acid or amino acid analogue and may be an L-amino acid, or a D-amino acid, or a methylated or an unmethylated amino acid
NFXCXFCXXXXCXXCX

SEQ ID NO: 95 - protein, 16 aa, Artificial Sequence
  Chemically Synthesized
  MISC_FEATURE (3)..(4): wherein x is a cysteine, penicillamine homocysteine, or 3-mercaptoproline
  MISC_FEATURE (5)..(6): wherein x is any natural, or unnatural amino acid or amino acid analogue and may be an L-amino acid, or a D-amino acid, or a methylated or an unmethylated amino acid
  MISC_FEATURE (7)..(8): wherein x is a cysteine, penicillamine homocysteine, or 3-mercaptoproline
  MISC_FEATURE (9)..(11): wherein x is any natural, or unnatural amino acid or amino acid analogue and may be an L-amino acid, or a D-amino acid, or a methylated or an unmethylated amino acid
  MISC_FEATURE (12)..(12): wherein x is a cysteine, penicillamine homocysteine, or 3-mercaptoproline
  MISC_FEATURE (13)..(14): wherein x is any natural, or unnatural amino acid or amino acid analogue and may be an L-amino acid, or a D-amino acid, or a methylated or an unmethylated amino acid
  MISC_FEATURE (15)..(15): wherein x is a cysteine, penicillamine homocysteine, or 3-mercaptoproline
  MISC_FEATURE (16)..(16): wherein x is any natural, or unnatural amino acid or amino acid analogue and may be an L-amino acid, or a D-amino acid, or a methylated or an unmethylated amino acid
NFXXXXXXXXXXXXXX

SEQ ID NO: 96 - protein, 14 aa, Artificial Sequence
  Chemically Synthesized
  MISC_FEATURE (1)..(2): wherein x is a cysteine, penicillamine homocysteine, or 3-mercaptoproline
  MISC_FEATURE (4)..(4): wherein x is any natural, or unnatural amino acid or amino acid analogue and may be an L-amino acid, or a D-amino acid, or a methylated or an unmethylated amino acid
  MISC_FEATURE (5)..(6): wherein x is a cysteine, penicillamine homocysteine, or 3-mercaptoproline
  MISC_FEATURE (10)..(10): wherein x is a cysteine, penicillamine homocysteine, or 3-mercaptoproline
  MISC_FEATURE (13)..(13): wherein x is a cysteine, penicillamine homocysteine, or 3-mercaptoproline
XXEXXXNPAXTGXY

SEQ ID NO: 97 - protein, 13 aa, Artificial Sequence
  Chemically Synthesized
  MISC_FEATURE (1)..(2): wherein x is a cysteine, or penicillamine, homocysteine, or 3-mercaptoproline
  MISC_FEATURE (4)..(4): wherein x is any natural, or unnatural amino acid or amino acid analogue and may be an L-amino acid, or a D-amino acid, or a methylated or an unmethylated amino acid
  MISC_FEATURE (5)..(6): wherein x is a cysteine, or penicillamine, homocysteine, or 3-mercaptoproline
  MISC_FEATURE (10)..(10): wherein x is a cysteine, or penicillamine, homocysteine, or 3-mercaptoproline
  MISC_FEATURE (13)..(13): wherein x is a cysteine, or penicillamine, homocysteine, or 3-mercaptoproline
XXEXXXNPAXTGX

SEQ ID NO: 98 - protein, 20 aa, Artificial Sequence
  Chemically Synthesized
  MISC_FEATURE (1)..(1): wherein x is any natural, or unnatural amino acid or amino acid analogue, and  may be zero or one residue in length, and may be an L-amino acid, or a D-amino acid, or a methylated or an unmethylated amino acid
  MISC_FEATURE (2)..(2): wherein x is any natural, or unnatural amino acid or amino acid analogue, and  may be zero or one residue in length, and may be an L-amino acid, or a D-amino acid, or a methylated or an unmethylated amino acid
  MISC_FEATURE (3)..(3): wherein x is any natural, or unnatural amino acid or amino acid analogue, and  may be zero or one residue in length, and may be an L-amino acid, or a D-amino acid, or a methylated or an unmethylated amino acid
  MISC_FEATURE (4)..(4): wherein x is any natural, or unnatural amino acid or amino acid analogue, and  may be zero or one residue in length, and may be an L-amino acid, or a D-amino acid, or a methylated or an unmethylated amino acid
  MISC_FEATURE (5)..(5): wherein x is any natural, or unnatural amino acid or amino acid analogue, and  may be zero or one residue in length, and may be an L-amino acid, or a D-amino acid, or a methylated or an unmethylated amino acid
  MISC_FEATURE (6)..(6): wherein x is any natural, or unnatural amino acid or amino acid analogue, and  may be zero or one residue in length, and may be an L-amino acid, or a D-amino acid, or a methylated or an unmethylated amino acid
  MISC_FEATURE (7)..(8): wherein x is a cysteine, penicillamine homocysteine, or 3-mercaptoproline
  MISC_FEATURE (9)..(10): wherein x is any natural, or unnatural amino acid or amino acid analogue and may be an L-amino acid, or a D-amino acid, or a methylated or an unmethylated amino acid
  MISC_FEATURE (11)..(12): wherein x is a cysteine, penicillamine homocysteine, or 3-mercaptoproline
  MISC_FEATURE (13)..(15): wherein x is any natural, or unnatural amino acid or amino acid analogue and may be an L-amino acid, or a D-amino acid, or a methylated or an unmethylated amino acid
  MISC_FEATURE (16)..(16): wherein x is a cysteine, penicillamine homocysteine, or 3-mercaptoproline
  MISC_FEATURE (17)..(18): wherein x is any natural, or unnatural amino acid or amino acid analogue and may be an L-amino acid, or a D-amino acid, or a methylated or an unmethylated amino acid
  MISC_FEATURE (19)..(19): wherein x is a cysteine, penicillamine homocysteine, or 3-mercaptoproline
  MISC_FEATURE (20)..(20): wherein x is any natural, or unnatural amino acid or amino acid analogue, and may be zero or one residue in length, and may be an L-amino acid, or a D-amino acid, or a methylated or an unmethylated amino acid
XXXXXXXXXXXXXXXXXXXX

SEQ ID NO: 99 - protein, 16 aa, Artificial Sequence
  Chemically Synthesized
  MISC_FEATURE (1)..(1): wherein ASN is a D-amino acid
  MISC_FEATURE (16)..(16): wherein LEU is a D-amino acid
  MISC_FEATURE (16)..(16): wherein LEU is conjugated to an AMIDE
NDECELCVNVACTGCL

SEQ ID NO: 100 - protein, 16 aa, Artificial Sequence
  Chemically Synthesized
  MISC_FEATURE (1)..(1): wherein ASN is a D-amino acid
  MISC_FEATURE (16)..(16): wherein SER is a D-amino acid
NDECELCVNVACTGCS

SEQ ID NO: 101 - protein, 16 aa, Artificial Sequence
  Chemically Synthesized
  MISC_FEATURE (1)..(1): wherein ASN is a D-amino acid
  MISC_FEATURE (16)..(16): wherein SER is a D-amino acid
  MISC_FEATURE (16)..(16): wherein SER is conjugated to an AMIDE
NDECELCVNVACTGCS

SEQ ID NO: 102 - protein, 16 aa, Artificial Sequence
  Chemically Synthesized
  MISC_FEATURE (1)..(1): wherein ASN is a D-amino acid
  MISC_FEATURE (16)..(16): wherein TYR is a D-amino acid
NDECELCVNVACTGCY

SEQ ID NO: 103 - protein, 16 aa, Artificial Sequence
  Chemically Synthesized
  MISC_FEATURE (1)..(1): wherein ASN is a D-amino acid
  MISC_FEATURE (16)..(16): wherein TYR is a D-amino acid
  MISC_FEATURE (16)..(16): wherein TYR is conjugated to an AMIDE
NDECELCVNVACTGCY

SEQ ID NO: 104 - protein, 16 aa, Artificial Sequence
  Chemically Synthesized
  MISC_FEATURE (1)..(1): wherein x is Pyroglutamic acid
  MISC_FEATURE (16)..(16): wherein LEU is conjugated to an AMIDE
  MISC_FEATURE (16)..(16): wherein LEU is a D-amino acid
XDECELCVNVACTGCL

SEQ ID NO: 105 - protein, 16 aa, Artificial Sequence
  Chemically Synthesized
  MISC_FEATURE (1)..(1): wherein ASN is attached to polyethylene glycol
  MISC_FEATURE (16)..(16): wherein LEU is attached to polyethylene glycol
NDECELCVNVACTGCL

SEQ ID NO: 106 - protein, 16 aa, Artificial Sequence
  Chemically Synthesized
  MISC_FEATURE (1)..(1): wherein ASN is attached to polyethylene glycol
NDECELCVNVACTGCL

SEQ ID NO: 107 - protein, 16 aa, Artificial Sequence
  Chemically Synthesized
  MISC_FEATURE (16)..(16): wherein LEU is attached to polyethylene glycol
NDECELCVNVACTGCL

SEQ ID NO: 108 - protein, 16 aa, Artificial Sequence
  Chemically Synthesized
  MISC_FEATURE (1)..(3): wherein x is any natural, or unnatural amino acid or amino acid analogue and may be an L-amino acid, or a D-amino acid, or a methylated or an unmethylated amino acid
  MISC_FEATURE (4)..(4): wherein x is a cysteine, penicillamine homocysteine, or 3-mercaptoproline
  MISC_FEATURE (5)..(6): wherein x is any natural, or unnatural amino acid or amino acid analogue, and may be an L-amino acid, or a D-amino acid, or a methylated or an unmethylated amino acid
  MISC_FEATURE (7)..(7): wherein x is a cysteine, penicillamine homocysteine, or 3-mercaptoproline
  MISC_FEATURE (8)..(11): wherein x is any natural, or unnatural amino acid or amino acid analogue, and may be an L-amino acid, or a D-amino acid, or a methylated or an unmethylated amino acid
  MISC_FEATURE (12)..(12): wherein x is a cysteine, penicillamine homocysteine, or 3-mercaptoproline
  MISC_FEATURE (13)..(14): wherein x is any natural, or unnatural amino acid or amino acid analogue, and may be an L-amino acid, or a D-amino acid, or a methylated or an unmethylated amino acid
  MISC_FEATURE (15)..(15): wherein x is a cysteine, penicillamine homocysteine, or 3-mercaptoproline
  MISC_FEATURE (16)..(16): wherein x is any natural, or unnatural amino acid or amino acid analogue, and may be an L-amino acid, or a D-amino acid, or a methylated or an unmethylated amino acid
XXXXXXXXXXXXXXXX

SEQ ID NO: 109 - protein, 16 aa, Artificial Sequence
  Chemically Synthesized
NDDCELCVNVACTGCL

SEQ ID NO: 110 - protein, 16 aa, Artificial Sequence
  Chemically Synthesized
EDDCELCVNVACTGCL

SEQ ID NO: 111 - protein, 16 aa, Artificial Sequence
  Chemically Synthesized
EDECELCVNVACTGCL

SEQ ID NO: 112 - protein, 16 aa, Artificial Sequence
  Chemically Synthesized
EEDCELCVNVACTGCL

SEQ ID NO: 113 - protein, 16 aa, Artificial Sequence
  Chemically Synthesized
EEECELCVNVACTGCL

SEQ ID NO: 114 - protein, 16 aa, Artificial Sequence
  Chemically Synthesized
DDDCELCVNVACTGCL

SEQ ID NO: 115 - protein, 16 aa, Artificial Sequence
  Chemically Synthesized
DDECELCVNVACTGCL

SEQ ID NO: 116 - protein, 16 aa, Artificial Sequence
  Chemically Synthesized
DEDCELCVNVACTGCL

SEQ ID NO: 117 - protein, 16 aa, Artificial Sequence
  Chemically Synthesized
DEECELCVNVACTGCL

SEQ ID NO: 118 - protein, 16 aa, Artificial Sequence
  Chemically Synthesized
QDDCELCVNVACTGCL

SEQ ID NO: 119 - protein, 16 aa, Artificial Sequence
  Chemically Synthesized
QDECELCVNVACTGCL

SEQ ID NO: 120 - protein, 16 aa, Artificial Sequence
  Chemically Synthesized
QEDCELCVNVACTGCL

SEQ ID NO: 121 - protein, 16 aa, Artificial Sequence
  Chemically Synthesized
QEECELCVNVACTGCL

SEQ ID NO: 122 - protein, 16 aa, Artificial Sequence
  Chemically Synthesized
KDDCELCVNVACTGCL

SEQ ID NO: 123 - protein, 16 aa, Artificial Sequence
  Chemically Synthesized
KDECELCVNVACTGCL

SEQ ID NO: 124 - protein, 16 aa, Artificial Sequence
  Chemically Synthesized
KEDCELCVNVACTGCL

SEQ ID NO: 125 - protein, 16 aa, Artificial Sequence
  Chemically Synthesized
KEECELCVNVACTGCL

SEQ ID NO: 126 - protein, 16 aa, Artificial Sequence
  Chemically Synthesized
EDDCELCVNVACTGCS

SEQ ID NO: 127 - protein, 16 aa, Artificial Sequence
  Chemically Synthesized
EDECELCVNVACTGCS

SEQ ID NO: 128 - protein, 16 aa, Artificial Sequence
  Chemically Synthesized
EEDCELCVNVACTGCS

SEQ ID NO: 129 - protein, 16 aa, Artificial Sequence
  Chemically Synthesized
EEECELCVNVACTGCS

SEQ ID NO: 130 - protein, 16 aa, Artificial Sequence
  Chemically Synthesized
DDDCELCVNVACTGCS

SEQ ID NO: 131 - protein, 16 aa, Artificial Sequence
  Chemically Synthesized
DDECELCVNVACTGCS

SEQ ID NO: 132 - protein, 16 aa, Artificial Sequence
  Chemically Synthesized
DEDCELCVNVACTGCS

SEQ ID NO: 133 - protein, 16 aa, Artificial Sequence
  Chemically Synthesized
DEECELCVNVACTGCS

SEQ ID NO: 134 - protein, 16 aa, Artificial Sequence
  Chemically Synthesized
QDDCELCVNVACTGCS

SEQ ID NO: 135 - protein, 16 aa, Artificial Sequence
  Chemically Synthesized
QDECELCVNVACTGCS

SEQ ID NO: 136 - protein, 16 aa, Artificial Sequence
  Chemically Synthesized
QEDCELCVNVACTGCS

SEQ ID NO: 137 - protein, 16 aa, Artificial Sequence
  Chemically Synthesized
QEECELCVNVACTGCS

SEQ ID NO: 138 - protein, 16 aa, Artificial Sequence
  Chemically Synthesized
KDDCELCVNVACTGCS

SEQ ID NO: 139 - protein, 16 aa, Artificial Sequence
  Chemically Synthesized
KDECELCVNVACTGCS

SEQ ID NO: 140 - protein, 16 aa, Artificial Sequence
  Chemically Synthesized
KEDCELCVNVACTGCS

SEQ ID NO: 141 - protein, 16 aa, Artificial Sequence
  Chemically Synthesized
KEECELCVNVACTGCS

SEQ ID NO: 142 - protein, 16 aa, Artificial Sequence
  Chemically Synthesized
EDDCELCINMACTGCL

SEQ ID NO: 143 - protein, 16 aa, Artificial Sequence
  Chemically Synthesized
EDECELCINMACTGCL

SEQ ID NO: 144 - protein, 16 aa, Artificial Sequence
  Chemically Synthesized
EEDCELCINMACTGCL

SEQ ID NO: 145 - protein, 16 aa, Artificial Sequence
  Chemically Synthesized
EEECELCINMACTGCL

SEQ ID NO: 146 - protein, 16 aa, Artificial Sequence
  Chemically Synthesized
DDDCELCINMACTGCL

SEQ ID NO: 147 - protein, 16 aa, Artificial Sequence
  Chemically Synthesized
DDECELCINMACTGCL

SEQ ID NO: 148 - protein, 16 aa, Artificial Sequence
  Chemically Synthesized
DEDCELCINMACTGCL

SEQ ID NO: 149 - protein, 16 aa, Artificial Sequence
  Chemically Synthesized
DEECELCINMACTGCL

SEQ ID NO: 150 - protein, 16 aa, Artificial Sequence
  Chemically Synthesized
QDDCELCINMACTGCL

SEQ ID NO: 151 - protein, 16 aa, Artificial Sequence
  Chemically Synthesized
QDECELCINMACTGCL

SEQ ID NO: 152 - protein, 16 aa, Artificial Sequence
  Chemically Synthesized
QEDCELCINMACTGCL

SEQ ID NO: 153 - protein, 16 aa, Artificial Sequence
  Chemically Synthesized
QEECELCINMACTGCL

SEQ ID NO: 154 - protein, 16 aa, Artificial Sequence
  Chemically Synthesized
KDDCELCINMACTGCL

SEQ ID NO: 155 - protein, 16 aa, Artificial Sequence
  Chemically Synthesized
KDECELCINMACTGCL

SEQ ID NO: 156 - protein, 16 aa, Artificial Sequence
  Chemically Synthesized
KEDCELCINMACTGCL

SEQ ID NO: 157 - protein, 16 aa, Artificial Sequence
  Chemically Synthesized
KEECELCINMACTGCL

SEQ ID NO: 158 - protein, 16 aa, Artificial Sequence
  Chemically Synthesized
EDDCELCINMACTGCS

SEQ ID NO: 159 - protein, 16 aa, Artificial Sequence
  Chemically Synthesized
EDECELCINMACTGCS

SEQ ID NO: 160 - protein, 16 aa, Artificial Sequence
  Chemically Synthesized
EEDCELCINMACTGCS

SEQ ID NO: 161 - protein, 16 aa, Artificial Sequence
  Chemically Synthesized
EEECELCINMACTGCS

SEQ ID NO: 162 - protein, 16 aa, Artificial Sequence
  Chemically Synthesized
DDDCELCINMACTGCS

SEQ ID NO: 163 - protein, 16 aa, Artificial Sequence
  Chemically Synthesized
DDECELCINMACTGCS

SEQ ID NO: 164 - protein, 16 aa, Artificial Sequence
  Chemically Synthesized
DEDCELCINMACTGCS

SEQ ID NO: 165 - protein, 16 aa, Artificial Sequence
  Chemically Synthesized
DEECELCINMACTGCS

SEQ ID NO: 166 - protein, 16 aa, Artificial Sequence
  Chemically Synthesized
QDDCELCINMACTGCS

SEQ ID NO: 167 - protein, 16 aa, Artificial Sequence
  Chemically Synthesized
QDECELCINMACTGCS

SEQ ID NO: 168 - protein, 16 aa, Artificial Sequence
  Chemically Synthesized
QEDCELCINMACTGCS

SEQ ID NO: 169 - protein, 16 aa, Artificial Sequence
  Chemically Synthesized
QEECELCINMACTGCS

SEQ ID NO: 170 - protein, 16 aa, Artificial Sequence
  Chemically Synthesized
KDDCELCINMACTGCS

SEQ ID NO: 171 - protein, 16 aa, Artificial Sequence
  Chemically Synthesized
KDECELCINMACTGCS

SEQ ID NO: 172 - protein, 16 aa, Artificial Sequence
  Chemically Synthesized
KEDCELCINMACTGCS

SEQ ID NO: 173 - protein, 16 aa, Artificial Sequence
  Chemically Synthesized
KEECELCINMACTGCS

SEQ ID NO: 174 - protein, 15 aa, Artificial Sequence
  Chemically Synthesized
  MISC_FEATURE (1)..(3): wherein x is any natural, or unnatural amino acid, or amino acid analogue, and may be an L-amino acid, or a D-amino acid, or a methylated or an unmethylated amino acid
  MISC_FEATURE (4)..(4): wherein x is a cysteine, penicillamine homocysteine, or 3-mercaptoproline
  MISC_FEATURE (5)..(6): wherein x is any natural, or unnatural amino acid, or amino acid analogue, and may be an L-amino acid, or a D-amino acid, or a methylated or an unmethylated amino acid
  MISC_FEATURE (7)..(7): wherein x is a cysteine, penicillamine homocysteine, or 3-mercaptoproline
  MISC_FEATURE (8)..(11): wherein x is any natural, or unnatural amino acid, or amino acid analogue, and may be an L-amino acid, or a D-amino acid, or a methylated or an unmethylated amino acid
  MISC_FEATURE (12)..(12): wherein x is a cysteine, penicillamine homocysteine, or 3-mercaptoproline
  MISC_FEATURE (13)..(14): wherein x is any natural, or unnatural amino acid, or amino acid analogue, and may be an L-amino acid, or a D-amino acid, or a methylated or an unmethylated amino acid
  MISC_FEATURE (15)..(15): wherein x is a cysteine, penicillamine homocysteine, or 3-mercaptoproline
XXXXXXXXXXXXXXX

SEQ ID NO: 175 - protein, 15 aa, Artificial Sequence
  Chemically Synthesized
SHTCEICAFAACAGC

SEQ ID NO: 176 - protein, 15 aa, Artificial Sequence
  Chemically Synthesized
SHTCEICANAACAGC

SEQ ID NO: 177 - protein, 15 aa, Artificial Sequence
  Chemically Synthesized
SHTCELCANAACAGC

SEQ ID NO: 178 - protein, 15 aa, Artificial Sequence
  Chemically Synthesized
SHTCEVCANAACAGC

SEQ ID NO: 179 - protein, 15 aa, Artificial Sequence
  Chemically Synthesized
SHTCEYCANAACAGC

SEQ ID NO: 180 - protein, 15 aa, Artificial Sequence
  Chemically Synthesized
SHTCEICANAACAGC

SEQ ID NO: 181 - protein, 15 aa, Artificial Sequence
  Chemically Synthesized
SHTCELCANAACAGC

SEQ ID NO: 182 - protein, 15 aa, Artificial Sequence
  Chemically Synthesized
SHTCEVCANAACAGC

SEQ ID NO: 183 - protein, 15 aa, Artificial Sequence
  Chemically Synthesized
SHTCEYCANAACAGC

SEQ ID NO: 184 - protein, 15 aa, Artificial Sequence
  Chemically Synthesized
SHTCEICANAACAGC

SEQ ID NO: 185 - protein, 15 aa, Artificial Sequence
  Chemically Synthesized
SHTCELCANAACAGC

SEQ ID NO: 186 - protein, 15 aa, Artificial Sequence
  Chemically Synthesized
SHTCEVCANAACAGC

SEQ ID NO: 187 - protein, 15 aa, Artificial Sequence
  Chemically Synthesized
SHTCEYCANAACAGC

SEQ ID NO: 188 - protein, 15 aa, Artificial Sequence
  Chemically Synthesized
SHTCEICANAACAGC

SEQ ID NO: 189 - protein, 15 aa, Artificial Sequence
  Chemically Synthesized
SHTCELCANAACAGC

SEQ ID NO: 190 - protein, 15 aa, Artificial Sequence
  Chemically Synthesized
SHTCEVCANAACAGC

SEQ ID NO: 191 - protein, 15 aa, Artificial Sequence
  Chemically Synthesized
SHTCEYCANAACAGC

SEQ ID NO: 192 - protein, 15 aa, Artificial Sequence
  Chemically Synthesized
NDECEICANAACAGC

SEQ ID NO: 193 - protein, 15 aa, Artificial Sequence
  Chemically Synthesized
NDECELCANAACAGC

SEQ ID NO: 194 - protein, 15 aa, Artificial Sequence
  Chemically Synthesized
NDECEVCANAACAGC

SEQ ID NO: 195 - protein, 15 aa, Artificial Sequence
  Chemically Synthesized
NDECEYCANAACAGC

SEQ ID NO: 196 - protein, 15 aa, Artificial Sequence
  Chemically Synthesized
NDECEICANAACAGC

SEQ ID NO: 197 - protein, 15 aa, Artificial Sequence
  Chemically Synthesized
NDECELCANAACAGC

SEQ ID NO: 198 - protein, 15 aa, Artificial Sequence
  Chemically Synthesized
NDECEVCANAACAGC

SEQ ID NO: 199 - protein, 15 aa, Artificial Sequence
  Chemically Synthesized
NDECEYCANAACAGC

SEQ ID NO: 200 - protein, 15 aa, Artificial Sequence
  Chemically Synthesized
NDECEICANAACAGC

SEQ ID NO: 201 - protein, 15 aa, Artificial Sequence
  Chemically Synthesized
NDECELCANAACAGC

SEQ ID NO: 202 - protein, 15 aa, Artificial Sequence
  Chemically Synthesized
NDECEVCANAACAGC

SEQ ID NO: 203 - protein, 15 aa, Artificial Sequence
  Chemically Synthesized
NDECEYCANAACAGC

SEQ ID NO: 204 - protein, 15 aa, Artificial Sequence
  Chemically Synthesized
NDECEICANAACAGC

SEQ ID NO: 205 - protein, 15 aa, Artificial Sequence
  Chemically Synthesized
NDECELCANAACAGC

SEQ ID NO: 206 - protein, 15 aa, Artificial Sequence
  Chemically Synthesized
NDECEVCANAACAGC

SEQ ID NO: 207 - protein, 15 aa, Artificial Sequence
  Chemically Synthesized
NDECEYCANAACAGC

SEQ ID NO: 208 - protein, 17 aa, Artificial Sequence
  Chemically Synthesized
  MISC_FEATURE (1)..(3): wherein x is any natural, or unnatural amino acid, or amino acid analogue, and may be an L-amino acid, or a D-amino acid, or a methylated, or an unmethylated amino acid
  MISC_FEATURE (4)..(4): wherein x is a cysteine, penicillamine homocysteine, or 3-mercaptoproline
  MISC_FEATURE (5)..(6): wherein x is any natural, or unnatural amino acid, or amino acid analogue, and may be an L-amino acid, or a D-amino acid, or a methylated, or an unmethylated amino acid
  MISC_FEATURE (7)..(7): wherein x is a cysteine, penicillamine homocysteine, or 3-mercaptoproline
  MISC_FEATURE (8)..(11): wherein x is any natural, or unnatural amino acid, or amino acid analogue, and may be an L-amino acid, or a D-amino acid, or a methylated, or an unmethylated amino acid
  MISC_FEATURE (12)..(12): wherein x is a cysteine, penicillamine homocysteine, or 3-mercaptoproline
  MISC_FEATURE (13)..(14): wherein x is any natural, or unnatural amino acid, or amino acid analogue, and may be an L-amino acid, or a D-amino acid, or a methylated, or an unmethylated amino acid
  MISC_FEATURE (15)..(15): wherein x is any natural, or unnatural amino acid, or amino acid analogue and may be an L-amino acid, or a D-amino acid, or a methylated, or an unmethylated amino acid
  MISC_FEATURE (16)..(16): wherein x is any natural, or unnatural amino acid, or amino acid analogue, and may be zero or one residue in length, and may be an L-amino acid, or a D-amino acid, or a methylated, or an unmethylated amino acid
  MISC_FEATURE (17)..(17): wherein x is any natural, or unnatural amino acid, or amino acid analogue, and may be zero or one residue in length, and may be an L-amino acid, or a D-amino acid, or a methylated, or an unmethylated amino acid
XXXXXXXXXXXXXXXXX

SEQ ID NO: 209 - protein, 15 aa, Artificial Sequence
  Chemically Synthesized
QEECELCINMACTGY

SEQ ID NO: 210 - protein, 15 aa, Artificial Sequence
  Chemically Synthesized
QEECETCINMACTGY

SEQ ID NO: 211 - protein, 15 aa, Artificial Sequence
  Chemically Synthesized
QDECETCINMACTGY

SEQ ID NO: 212 - protein, 15 aa, Artificial Sequence
  Chemically Synthesized
QDDCETCINMACTGY

SEQ ID NO: 213 - protein, 15 aa, Artificial Sequence
  Chemically Synthesized
QEDCETCINMACTGY

SEQ ID NO: 214 - protein, 15 aa, Artificial Sequence
  Chemically Synthesized
QEECEECINMACTGY

SEQ ID NO: 215 - protein, 15 aa, Artificial Sequence
  Chemically Synthesized
QDECEECINMACTGY

SEQ ID NO: 216 - protein, 15 aa, Artificial Sequence
  Chemically Synthesized
QDDCEECINMACTGY

SEQ ID NO: 217 - protein, 15 aa, Artificial Sequence
  Chemically Synthesized
QEDCEECINMACTGY

SEQ ID NO: 218 - protein, 15 aa, Artificial Sequence
  Chemically Synthesized
QEECEYCINMACTGY

SEQ ID NO: 219 - protein, 15 aa, Artificial Sequence
  Chemically Synthesized
QDECEYCINMACTGY

SEQ ID NO: 220 - protein, 15 aa, Artificial Sequence
  Chemically Synthesized
QDDCEYCINMACTGY

SEQ ID NO: 221 - protein, 15 aa, Artificial Sequence
  Chemically Synthesized
QEDCEYCINMACTGY

SEQ ID NO: 222 - protein, 15 aa, Artificial Sequence
  Chemically Synthesized
QEECEICINMACTGY

SEQ ID NO: 223 - protein, 15 aa, Artificial Sequence
  Chemically Synthesized
QDECEICINMACTGY

SEQ ID NO: 224 - protein, 15 aa, Artificial Sequence
  Chemically Synthesized
QDDCEICINMACTGY

SEQ ID NO: 225 - protein, 15 aa, Artificial Sequence
  Chemically Synthesized
QEDCEICINMACTGY

SEQ ID NO: 226 - protein, 16 aa, Artificial Sequence
  Chemically Synthesized
QEECETCINMACTGCS

SEQ ID NO: 227 - protein, 16 aa, Artificial Sequence
  Chemically Synthesized
QDECETCINMACTGCS

SEQ ID NO: 228 - protein, 16 aa, Artificial Sequence
  Chemically Synthesized
QDDCETCINMACTGCS

SEQ ID NO: 229 - protein, 16 aa, Artificial Sequence
  Chemically Synthesized
QEDCETCINMACTGCS

SEQ ID NO: 230 - protein, 16 aa, Artificial Sequence
  Chemically Synthesized
QEECEECINMACTGCS

SEQ ID NO: 231 - protein, 16 aa, Artificial Sequence
  Chemically Synthesized
QDECEECINMACTGCS

SEQ ID NO: 232 - protein, 16 aa, Artificial Sequence
  Chemically Synthesized
QDDCEECINMACTGCS

SEQ ID NO: 233 - protein, 16 aa, Artificial Sequence
  Chemically Synthesized
QEDCEECINMACTGCS

SEQ ID NO: 234 - protein, 16 aa, Artificial Sequence
  Chemically Synthesized
QEECEYCINMACTGCS

SEQ ID NO: 235 - protein, 16 aa, Artificial Sequence
  Chemically Synthesized
QDECEYCINMACTGCS

SEQ ID NO: 236 - protein, 16 aa, Artificial Sequence
  Chemically Synthesized
QDDCEYCINMACTGCS

SEQ ID NO: 237 - protein, 16 aa, Artificial Sequence
  Chemically Synthesized
QEDCEYCINMACTGCS

SEQ ID NO: 238 - protein, 16 aa, Artificial Sequence
  Chemically Synthesized
QEECEICINMACTGCS

SEQ ID NO: 239 - protein, 16 aa, Artificial Sequence
  Chemically Synthesized
QDECEICINMACTGCS

SEQ ID NO: 240 - protein, 16 aa, Artificial Sequence
  Chemically Synthesized
QDDCEICINMACTGCS

SEQ ID NO: 241 - protein, 16 aa, Artificial Sequence
  Chemically Synthesized
QEDCEICINMACTGCS

SEQ ID NO: 242 - protein, 22 aa, Artificial Sequence
  Chemically Synthesized
NSSNSSNYCCEKCCNPACTGCY

SEQ ID NO: 243 - protein, 16 aa, Artificial Sequence
  Chemically Synthesized
  MISC_FEATURE (1)..(1): wherein ASN is attached to polyethylene glycol
  MISC_FEATURE (16)..(16): wherein TYR is attached to polyethylene glycol
NFCCETCCNPACTGCY

SEQ ID NO: 244 - protein, 16 aa, Artificial Sequence
  Chemically Synthesized
  MISC_FEATURE (1)..(1): wherein ASN is attached to polyethylene glycol
NFCCETCCNPACTGCY

SEQ ID NO: 245 - protein, 16 aa, Artificial Sequence
  Chemically Synthesized
  MISC_FEATURE (16)..(16): wherein TYR is attached to polyethylene glycol
NFCCETCCNPACTGCY

SEQ ID NO: 246 - protein, 16 aa, Artificial Sequence
  Chemically Synthesized
NFCCEYCCNPACTGCY

SEQ ID NO: 247 - protein, 16 aa, Artificial Sequence
  Chemically Synthesized
  MISC_FEATURE (1)..(1): wherein ASN is a D-amino acid
  MISC_FEATURE (16)..(16): wherein TYR is a D-amino acid
NFCCEYCCNPACTGCY

SEQ ID NO: 248 - protein, 16 aa, Artificial Sequence
  Chemically Synthesized
  MISC_FEATURE (16)..(16): wherein TYR is a D-amino acid
NFCCEYCCNPACTGCY

SEQ ID NO: 249 - protein, 16 aa, Artificial Sequence
  Chemically Synthesized
  MISC_FEATURE (1)..(1): wherein ASN is a D-amino acid
NFCCEYCCNPACTGCY

SEQ ID NO: 250 - protein, 34 aa, Artificial Sequence
  Chemically Synthesized
IKPEAPGEDASPEELNRYYASLRHYLNLVTRQRY

SEQ ID NO: 251 - protein, 27 aa, Artificial Sequence
  Chemically Synthesized
  MISC_FEATURE (1)..(1): wherein HIS is conjugated to an AMINE having the general formula R-NH, and wherein R is a hydrogen or an organic compound having one, two, three, four, five, six, seven, eight, nine, or ten carbon atoms
  MISC_FEATURE (27)..(27): wherein LYS is conjugated to an AMIDE
HAEGTFTSDVSYLEGQAAKEFIAWLVK

SEQ ID NO: 252 - protein, 5 aa, Artificial Sequence
  Chemically Synthesized Sialorphin-related polypeptide
QHNPR

SEQ ID NO: 253 - protein, 6 aa, Artificial Sequence
  Chemically Synthesized Sialorphin-related polypeptide
VQHNPR

SEQ ID NO: 254 - protein, 7 aa, Artificial Sequence
  Chemically Synthesized Sialorphin-related polypeptide
VRQHNPR

SEQ ID NO: 255 - protein, 8 aa, Artificial Sequence
  Chemically Synthesized Sialorphin-related polypeptide
VRGQHNPR

SEQ ID NO: 256 - protein, 9 aa, Artificial Sequence
  Chemically Synthesized Sialorphin-related polypeptide
VRGPQHNPR

SEQ ID NO: 257 - protein, 10 aa, Artificial Sequence
  Chemically Synthesized Sialorphin-related polypeptide
VRGPRQHNPR

SEQ ID NO: 258 - protein, 11 aa, Artificial Sequence
  Chemically Synthesized Sialorphin-related polypeptide
VRGPRRQHNPR

SEQ ID NO: 259 - protein, 6 aa, Artificial Sequence
  Chemically Synthesized Sialorphin-related polypeptide
RQHNPR

SEQ ID NO: 260 - protein, 5 aa, Artificial Sequence
  Chemically Synthesized Enkephalin Pentapeptide
  MISC_FEATURE (2)..(2): wherein LYS is a D-amino acid
  MISC_FEATURE (5)..(5): wherein x is a L-homoserine
YKGFX

SEQ ID NO: 261 - protein, 4 aa, Artificial Sequence
  Chemically Synthesized Frakefamide
  MISC_FEATURE (2)..(2): wherein ALA is a D-amino acid
  MOD_RES (3)..(3): wherein PHE is fluorinated at the phenyl group at 4-position
  MISC_FEATURE (4)..(4): wherein PHE is attached to an AMINE
YAFF